European Patent Application EP 4 545 565 A1, published April 30, 2025. Title: 结合EGFR和B7-H3的双特异性抗体. Applicant: 信达生物制药(苏州)有限公司. Application WO. The sequence listing filed with the application follows.

SEQUENCE LISTING (54 sequences)

SEQ ID NO: 1 - protein, 125 aa, artificial sequence [sequence omitted]

SEQ ID NO: 2 - protein, 107 aa, artificial sequence [sequence omitted]

SEQ ID NO: 3 - protein, 118 aa, artificial sequence
QVQLVQSGAEVKKPGASVKVSCKASGYTFTEYIMHWVRQAPGQRLEWMGGINPGTGGTTYNQKFKDRVTITVDTSASTAYMELSSLRSEDTAVYYCTRRTPPWHFAVWGQGTLVTVSS

SEQ ID NO: 4 - protein, 106 aa, artificial sequence
DIQLTQSPSFLSASVGDRVTITCSASSSVSYIHWYQQKPGKAPKRWIYDTSRLASGVPSRFSGSGSGTEFTLTISSLQPEDFATYYCQQWSSAPLTFGGGTKVEIK

SEQ ID NO: 5 - protein, 119 aa, artificial sequence
QVQLVQSGAEVKKPGASVKVSCKASGYIFTSYWIHWVRQAPGQGLEWMGRIYPGTESTFYNEKFKGRVTMTRDTSTSTVYMELSSLRSEDTAVYYCHFITASDWYFDVWGQGTLVTVSS

SEQ ID NO: 6 - protein, 108 aa, artificial sequence
EIVLTQSPATLSLSPGERATLSCSVSSSVQSNYLYWYQQKPGQAPRLLIYGTSNLASGIPARFSGSGSGTDFTLTISSLEPEDFAVYYCYQWSSYPFTFGQGTKLEIK

SEQ ID NO: 7 - protein, 117 aa, artificial sequence
QVQLVQSGAEVKKPGSSVKVSCKASGYTFSDYVISWVRQAPGQGLEWMGEIYPRGGIIHYNEKFKARVTITADKSTSTAYMELSSLRSEDTAVYYCARLWDWYFDVWGQGTLVTVSS

SEQ ID NO: 8 - protein, 113 aa, artificial sequence
EIVLTQSPGTLSLSPGERATLSCRSSQSLVHSQGITYLDWYQQKPGQAPRLLIYKVSNRFSGIPDRFSGSGSGTDFTLTISRLEPEDFAVYYCSQGTHVPPWTFGGGTKVEIK

SEQ ID NO: 9 - protein, 5 aa, artificial sequence
TYGMH

SEQ ID NO: 10 - protein, 17 aa, artificial sequence
VIWDDGSYKYYGDSVKG

SEQ ID NO: 11 - protein, 13 aa, artificial sequence
DGITMVRGVMKDY

SEQ ID NO: 12 - protein, 11 aa, artificial sequence
RASQDISSALV

SEQ ID NO: 13 - protein, 7 aa, artificial sequence
DASSLES

SEQ ID NO: 14 - protein, 9 aa, artificial sequence
QQFNSYPLT

SEQ ID NO: 15 - protein, 10 aa, artificial sequence
GYTFTEYIMH

SEQ ID NO: 16 - protein, 17 aa, artificial sequence
GINPGTGGTTYNQKFKD

SEQ ID NO: 17 - protein, 9 aa, artificial sequence
RTPPWHFAV

SEQ ID NO: 18 - protein, 10 aa, artificial sequence
SASSSVSYIH

SEQ ID NO: 19 - protein, 7 aa, artificial sequence
DTSRLAS

SEQ ID NO: 20 - protein, 9 aa, artificial sequence
QQWSSAPLT

SEQ ID NO: 21 - protein, 10 aa, artificial sequence
GYIFTSYWIH

SEQ ID NO: 22 - protein, 17 aa, artificial sequence
RIYPGTESTFYNEKFKG

SEQ ID NO: 23 - protein, 10 aa, artificial sequence
ITASDWYFDV

SEQ ID NO: 24 - protein, 12 aa, artificial sequence
SVSSSVQSNYLY

SEQ ID NO: 25 - protein, 7 aa, artificial sequence
GTSNLAS

SEQ ID NO: 26 - protein, 9 aa, artificial sequence
YQWSSYPFT

SEQ ID NO: 27 - protein, 10 aa, artificial sequence
GYTFSDYVIS

SEQ ID NO: 28 - protein, 17 aa, artificial sequence
EIYPRGGIIHYNEKFKA

SEQ ID NO: 29 - protein, 10 aa, artificial sequence
ARLWDWYFDV

SEQ ID NO: 30 - protein, 16 aa, artificial sequence
RSSQSLVHSQGITYLD

SEQ ID NO: 31 - protein, 7 aa, artificial sequence
KVSNRFS

SEQ ID NO: 32 - protein, 10 aa, artificial sequence
SQGTHVPPWT

SEQ ID NO: 33 - protein, 455 aa, artificial sequence
QVQLVESGGGVVQPGRSLRLSCAASGFTFSTYGMHWVRQAPGKGLEWVAVIWDDGSYKYYGDSVKGRFTISRDNSKNTLYLQMNSLRAEDTAVYYCARDGITMVRGVMKDYFDYWGQGTLVTVSSASTKGPSVFPLAPSSKSTSGGTAALGCLVKDYFPEPVTVSWNSGALTSGVHTFPAVLQSSGLYSLSSVVTVPSSSLGTQTYICNVNHKPSNTKVDKKVEPKSCDKTHTCPPCPAPELLGGPSVFLFPPKPKDTLMISRTPEVTCVVVDVSHEDPEVKFNWYVDGVEVHNAKTKPREEQYNSTYRVVSVLTVLHQDWLNGKEYKCKVSNKALPAPIEKTISKAKGQPREPQVTTLPPSRDELTKNQVSLTCLVSGFYPSDIAVEWESNGQPENNYKTTPPVLDSDGSFFLYSDLTVDKSRWQQGNVFSCSVMHEALHNHYTQKSLSLSPGK

SEQ ID NO: 34 - protein, 214 aa, artificial sequence
AIQLTQSPSSLSASVGDRVTITCRASQDISSALVWYQQKPGKAPKLLIYDASSLESGVPSRFSGSESGTDFTLTISSLQPEDFATYYCQQFNSYPLTFGGGTKVEIKRTVAAPSVFIFPPSDEQLKSGTASVVCLLNNFYPREAKVQWKVDNALQSGNSQESVTEQDSKDSTYSLSSTLTLSKADYEKHKVYACEVTHQGLSSPVTKSFNRGEC

SEQ ID NO: 35 - protein, 448 aa, artificial sequence
QVQLVQSGAEVKKPGASVKVSCKASGYTFTEYIMHWVRQAPGQRLEWMGGINPGTGGTTYNQKFKDRVTITVDTSASTAYMELSSLRSEDTAVYYCTRRTPPWHFAVWGQGTLVTVSSASTKGPSVFPLAPSSKSTSGGTAALGCLVKDYFPEPVTVSWNSGALTSGVHTFPAVLQSSGLYSLSSVVTVPSSSLGTQTYICNVNHKPSNTKVDKKVEPKSCDKTHTCPPCPAPELLGGPSVFLFPPKPKDTLMISRTPEVTCVVVDVSHEDPEVKFNWYVDGVEVHNAKTKPREEQYNSTYRVVSVLTVLHQDWLNGKEYKCKVSNKALPAPIEKTISKAKGQPREPQVYTLPPSRDELTKNQVRLTCLVKGFYPSDIAVEWESNGQPENNYKTTPPVLKSDGSFFLYSKLTVDKSRWQQGNVFSCSVMHEALHNHYTQKSLSLSPGK

SEQ ID NO: 36 - protein, 213 aa, artificial sequence
DIQLTQSPSFLSASVGDRVTITCSASSSVSYIHWYQQKPGKAPKRWIYDTSRLASGVPSRFSGSGSGTEFTLTISSLQPEDFATYYCQQWSSAPLTFGGGTKVEIKRTVAAPSVFIFPPSDEQLKSGTASVVCLLNNFYPREAKVQWKVDNALQSGNSQESVTEQDSKDSTYSLSSTLTLSKADYEKHKVYACEVTHQGLSSPVTKSFNRGEC

SEQ ID NO: 37 - protein, 449 aa, artificial sequence
QVQLVQSGAEVKKPGASVKVSCKASGYIFTSYWIHWVRQAPGQGLEWMGRIYPGTESTFYNEKFKGRVTMTRDTSTSTVYMELSSLRSEDTAVYYCHFITASDWYFDVWGQGTLVTVSSASTKGPSVFPLAPSSKSTSGGTAALGCLVKDYFPEPVTVSWNSGALTSGVHTFPAVLQSSGLYSLSSVVTVPSSSLGTQTYICNVNHKPSNTKVDKKVEPKSCDKTHTCPPCPAPELLGGPSVFLFPPKPKDTLMISRTPEVTCVVVDVSHEDPEVKFNWYVDGVEVHNAKTKPREEQYNSTYRVVSVLTVLHQDWLNGKEYKCKVSNKALPAPIEKTISKAKGQPREPQVYTLPPSRDELTKNQVRLTCLVKGFYPSDIAVEWESNGQPENNYKTTPPVLKSDGSFFLYSKLTVDKSRWQQGNVFSCSVMHEALHNHYTQKSLSLSPGK

SEQ ID NO: 38 - protein, 215 aa, artificial sequence
EIVLTQSPATLSLSPGERATLSCSVSSSVQSNYLYWYQQKPGQAPRLLIYGTSNLASGIPARFSGSGSGTDFTLTISSLEPEDFAVYYCYQWSSYPFTFGQGTKLEIKRTVAAPSVFIFPPSDEQLKSGTASVVCLLNNFYPREAKVQWKVDNALQSGNSQESVTEQDSKDSTYSLSSTLTLSKADYEKHKVYACEVTHQGLSSPVTKSFNRGEC

SEQ ID NO: 39 - protein, 447 aa, artificial sequence
QVQLVQSGAEVKKPGSSVKVSCKASGYTFSDYVISWVRQAPGQGLEWMGEIYPRGGIIHYNEKFKARVTITADKSTSTAYMELSSLRSEDTAVYYCARLWDWYFDVWGQGTLVTVSSASTKGPSVFPLAPSSKSTSGGTAALGCLVKDYFPEPVTVSWNSGALTSGVHTFPAVLQSSGLYSLSSVVTVPSSSLGTQTYICNVNHKPSNTKVDKKVEPKSCDKTHTCPPCPAPELLGGPSVFLFPPKPKDTLMISRTPEVTCVVVDVSHEDPEVKFNWYVDGVEVHNAKTKPREEQYNSTYRVVSVLTVLHQDWLNGKEYKCKVSNKALPAPIEKTISKAKGQPREPQVYTLPPSRDELTKNQVRLTCLVKGFYPSDIAVEWESNGQPENNYKTTPPVLKSDGSFFLYSKLTVDKSRWQQGNVFSCSVMHEALHNHYTQKSLSLSPGK

SEQ ID NO: 40 - protein, 220 aa, artificial sequence
EIVLTQSPGTLSLSPGERATLSCRSSQSLVHSQGITYLDWYQQKPGQAPRLLIYKVSNRFSGIPDRFSGSGSGTDFTLTISRLEPEDFAVYYCSQGTHVPPWTFGGGTKVEIKRTVAAPSVFIFPPSDEQLKSGTASVVCLLNNFYPREAKVQWKVDNALQSGNSQESVTEQDSKDSTYSLSSTLTLSKADYEKHKVYACEVTHQGLSSPVTKSFNRGEC

SEQ ID NO: 41 - protein, 304 aa, artificial sequence
MTQRLFVTGLSGFVGKHLQAYLAAAHTPWALLPVPHRYDLLEPDSLGDLWPELPDAVIHLAGQTYVPEAFRDPARTLQINLLGTLNLLQALKARGFSGTFLYISSGDVYGQVAEAALPIHEELIPHPRNPYAVSKLAAESLCLQWGITEGWRVLVARPFNHIGPGQKDSFVIASAARQIARMKQGLQANRLEVGDIDVSRDFLDVQDVLSAYLRLLSHGEAGAVYNVCSGQEQKIRELIELLADIAQVELEIVQDPARMRRAEQRRVRGSHARLHDTTGWKPEITIKQSLRAILSDWESRVREE

SEQ ID NO: 42 - protein, 98 aa, artificial sequence
ASTKGPSVFPLAPSSKSTSGGTAALGCLVKDYFPEPVTVSWNSGALTSGVHTFPAVLQSSGLYSLSSVVTVPSSSLGTQTYICNVNHKPSNTKVDKKV

SEQ ID NO: 43 - protein, 15 aa, artificial sequence
EPKSCDKTHTCPPCP

SEQ ID NO: 44 - protein, 110 aa, artificial sequence
APELLGGPSVFLFPPKPKDTLMISRTPEVTCVVVDVSHEDPEVKFNWYVDGVEVHNAKTKPREEQYNSTYRVVSVLTVLHQDWLNGKEYKCKVSNKALPAPIEKTISKAK

SEQ ID NO: 45 - protein, 107 aa, artificial sequence
GQPREPQVYTLPPSRDELTKNQVSLTCLVKGFYPSDIAVEWESNGQPENNYKTTPPVLDSDGSFFLYSKLTVDKSRWQQGNVFSCSVMHEALHNHYTQKSLSLSPGK

SEQ ID NO: 46 - protein, 217 aa, artificial sequence
APELLGGPSVFLFPPKPKDTLMISRTPEVTCVVVDVSHEDPEVKFNWYVDGVEVHNAKTKPREEQYNSTYRVVSVLTVLHQDWLNGKEYKCKVSNKALPAPIEKTISKAKGQPREPQVYTLPPSRDELTKNQVSLTCLVKGFYPSDIAVEWESNGQPENNYKTTPPVLDSDGSFFLYSKLTVDKSRWQQGNVFSCSVMHEALHNHYTQKSLSLSPGK

SEQ ID NO: 47 - protein, 232 aa, artificial sequence
EPKSCDKTHTCPPCPAPELLGGPSVFLFPPKPKDTLMISRTPEVTCVVVDVSHEDPEVKFNWYVDGVEVHNAKTKPREEQYNSTYRVVSVLTVLHQDWLNGKEYKCKVSNKALPAPIEKTISKAKGQPREPQVYTLPPSRDELTKNQVSLTCLVKGFYPSDIAVEWESNGQPENNYKTTPPVLDSDGSFFLYSKLTVDKSRWQQGNVFSCSVMHEALHNHYTQKSLSLSPGK

SEQ ID NO: 48 - protein, 107 aa, artificial sequence
GQPREPQVTTLPPSRDELTKNQVSLTCLVSGFYPSDIAVEWESNGQPENNYKTTPPVLDSDGSFFLYSDLTVDKSRWQQGNVFSCSVMHEALHNHYTQKSLSLSPGK

SEQ ID NO: 49 - protein, 217 aa, artificial sequence
APELLGGPSVFLFPPKPKDTLMISRTPEVTCVVVDVSHEDPEVKFNWYVDGVEVHNAKTKPREEQYNSTYRVVSVLTVLHQDWLNGKEYKCKVSNKALPAPIEKTISKAKGQPREPQVTTLPPSRDELTKNQVSLTCLVSGFYPSDIAVEWESNGQPENNYKTTPPVLDSDGSFFLYSDLTVDKSRWQQGNVFSCSVMHEALHNHYTQKSLSLSPGK

SEQ ID NO: 50 - protein, 232 aa, artificial sequence
EPKSCDKTHTCPPCPAPELLGGPSVFLFPPKPKDTLMISRTPEVTCVVVDVSHEDPEVKFNWYVDGVEVHNAKTKPREEQYNSTYRVVSVLTVLHQDWLNGKEYKCKVSNKALPAPIEKTISKAKGQPREPQVTTLPPSRDELTKNQVSLTCLVSGFYPSDIAVEWESNGQPENNYKTTPPVLDSDGSFFLYSDLTVDKSRWQQGNVFSCSVMHEALHNHYTQKSLSLSPGK

SEQ ID NO: 51 - protein, 107 aa, artificial sequence
GQPREPQVYTLPPSRDELTKNQVRLTCLVKGFYPSDIAVEWESNGQPENNYKTTPPVLKSDGSFFLYSKLTVDKSRWQQGNVFSCSVMHEALHNHYTQKSLSLSPGK

SEQ ID NO: 52 - protein, 217 aa, artificial sequence
APELLGGPSVFLFPPKPKDTLMISRTPEVTCVVVDVSHEDPEVKFNWYVDGVEVHNAKTKPREEQYNSTYRVVSVLTVLHQDWLNGKEYKCKVSNKALPAPIEKTISKAKGQPREPQVYTLPPSRDELTKNQVRLTCLVKGFYPSDIAVEWESNGQPENNYKTTPPVLKSDGSFFLYSKLTVDKSRWQQGNVFSCSVMHEALHNHYTQKSLSLSPGK

SEQ ID NO: 53 - protein, 232 aa, artificial sequence
EPKSCDKTHTCPPCPAPELLGGPSVFLFPPKPKDTLMISRTPEVTCVVVDVSHEDPEVKFNWYVDGVEVHNAKTKPREEQYNSTYRVVSVLTVLHQDWLNGKEYKCKVSNKALPAPIEKTISKAKGQPREPQVYTLPPSRDELTKNQVRLTCLVKGFYPSDIAVEWESNGQPENNYKTTPPVLKSDGSFFLYSKLTVDKSRWQQGNVFSCSVMHEALHNHYTQKSLSLSPGK

SEQ ID NO: 54 - protein, 107 aa, artificial sequence [sequence omitted]